European Patent Specification EP 4 200 443 B1, published April 10, 2024. Title: A method for the isolation of double strand breaks. Applicant: University College Cardiff Consultants Ltd Broken String Biosciences Limited. The sequence listing filed with the application follows.

SEQUENCE LISTING (111 sequences)

SEQ ID NO: 1 - DNA, 58 bp, Artificial Sequence
  Adaptor Sequence
gatcggaagagcgtcgtgtagggaaagagtgtagatctcggtggtcgccgtatcattc

SEQ ID NO: 2 - DNA, 58 bp, Artificial Sequence
  Adaptor Sequence
aatgatacggcgaccaccgagatctacactctttccctacacgacgctcttccgatct

SEQ ID NO: 3 - DNA, 33 bp, Artificial Sequence
  Adaptor Sequence
gatcggaagagcacacgtctgaactccagtcac

SEQ ID NO: 4 - DNA, 64 bp, Artificial Sequence
  Adaptor Sequence
  misc_feature (25)..(30): n is a, c, g, or t
caagcagaagacggcatacgagatnnnnnngtgactggagttcagacgtgtgctcttccgatct

SEQ ID NO: 5 - DNA, 64 bp, Artificial Sequence
  Adaptor Sequence
caagcagaagacggcatacgagatcgtgatgtgactggagttcagacgtgtgctcttccgatct

SEQ ID NO: 6 - DNA, 64 bp, Artificial Sequence
  Adaptor Sequence
caagcagaagacggcatacgagatacatcggtgactggagttcagacgtgtgctcttccgatct

SEQ ID NO: 7 - DNA, 64 bp, Artificial Sequence
  Adaptor Sequence
caagcagaagacggcatacgagatgcctaagtgactggagttcagacgtgtgctcttccgatct

SEQ ID NO: 8 - DNA, 64 bp, Artificial Sequence
  Adaptor Sequence
caagcagaagacggcatacgagattggtcagtgactggagttcagacgtgtgctcttccgatct

SEQ ID NO: 9 - DNA, 64 bp, Artificial Sequence
  Adaptor Sequence
caagcagaagacggcatacgagatcactgtgtgactggagttcagacgtgtgctcttccgatct

SEQ ID NO: 10 - DNA, 64 bp, Artificial Sequence
  Adaptor Sequence
caagcagaagacggcatacgagatattggcgtgactggagttcagacgtgtgctcttccgatct

SEQ ID NO: 11 - DNA, 64 bp, Artificial Sequence
  Adaptor Sequence
caagcagaagacggcatacgagatgatctggtgactggagttcagacgtgtgctcttccgatct

SEQ ID NO: 12 - DNA, 64 bp, Artificial Sequence
  Adaptor Sequence
caagcagaagacggcatacgagattcaagtgtgactggagttcagacgtgtgctcttccgatct

SEQ ID NO: 13 - DNA, 64 bp, Artificial Sequence
  Adaptor Sequence
caagcagaagacggcatacgagatctgatcgtgactggagttcagacgtgtgctcttccgatct

SEQ ID NO: 14 - DNA, 64 bp, Artificial Sequence
  Adaptor Sequence
caagcagaagacggcatacgagataagctagtgactggagttcagacgtgtgctcttccgatct

SEQ ID NO: 15 - DNA, 64 bp, Artificial Sequence
  Adaptor Sequence
caagcagaagacggcatacgagatgtagccgtgactggagttcagacgtgtgctcttccgatct

SEQ ID NO: 16 - DNA, 64 bp, Artificial Sequence
  Adaptor Sequence
caagcagaagacggcatacgagattacaaggtgactggagttcagacgtgtgctcttccgatct

SEQ ID NO: 17 - DNA, 66 bp, Artificial Sequence
  Adaptor Sequence
caagcagaagacggcatacgagattgttgactgtgactggagttcagacgtgtgctcttccgatct

SEQ ID NO: 18 - DNA, 66 bp, Artificial Sequence
  Adaptor Sequence
caagcagaagacggcatacgagatacggaactgtgactggagttcagacgtgtgctcttccgatct

SEQ ID NO: 19 - DNA, 66 bp, Artificial Sequence
  Adaptor Sequence
caagcagaagacggcatacgagattctgacatgtgactggagttcagacgtgtgctcttccgatct

SEQ ID NO: 20 - DNA, 66 bp, Artificial Sequence
  Adaptor Sequence
caagcagaagacggcatacgagatcgggacgggtgactggagttcagacgtgtgctcttccgatct

SEQ ID NO: 21 - DNA, 66 bp, Artificial Sequence
  Adaptor Sequence
caagcagaagacggcatacgagatgtgcggacgtgactggagttcagacgtgtgctcttccgatct

SEQ ID NO: 22 - DNA, 66 bp, Artificial Sequence
  Adaptor Sequence
caagcagaagacggcatacgagatcgtttcacgtgactggagttcagacgtgtgctcttccgatct

SEQ ID NO: 23 - DNA, 66 bp, Artificial Sequence
  Adaptor Sequence
caagcagaagacggcatacgagataaggccacgtgactggagttcagacgtgtgctcttccgatct

SEQ ID NO: 24 - DNA, 66 bp, Artificial Sequence
  Adaptor Sequence
caagcagaagacggcatacgagattccgaaacgtgactggagttcagacgtgtgctcttccgatct

SEQ ID NO: 25 - DNA, 66 bp, Artificial Sequence
  Adaptor Sequence
caagcagaagacggcatacgagattacgtacggtgactggagttcagacgtgtgctcttccgatct

SEQ ID NO: 26 - DNA, 66 bp, Artificial Sequence
  Adaptor Sequence
caagcagaagacggcatacgagatatccactcgtgactggagttcagacgtgtgctcttccgatct

SEQ ID NO: 27 - DNA, 66 bp, Artificial Sequence
  Adaptor Sequence
caagcagaagacggcatacgagatatatcagtgtgactggagttcagacgtgtgctcttccgatct

SEQ ID NO: 28 - DNA, 66 bp, Artificial Sequence
  Adaptor Sequence
caagcagaagacggcatacgagataaaggaatgtgactggagttcagacgtgtgctcttccgatct

SEQ ID NO: 29 - DNA, 20 bp, Artificial Sequence
  gRNA targeting EMX1
gagtccgagcagaagaagaa

SEQ ID NO: 30 - DNA, 24 bp, Artificial Sequence
  Adaptor Sequence - optionally not present
atctcgtatgccgtcttctgcttg

SEQ ID NO: 31 - DNA, 20 bp, Artificial Sequence
  Adaptor Sequence - optionally not present
tcggtggtcgccgtatcatt

SEQ ID NO: 32 - DNA, 24 bp, Artificial Sequence
  Adaptor Sequence
caagcagaagacggcatacgagat

SEQ ID NO: 33 - DNA, 34 bp, Artificial Sequence
  Adaptor Sequence
gtgactggagttcagacgtgtgctcttccgatct

SEQ ID NO: 34 - DNA, 20 bp, Artificial Sequence
  Adaptor Sequence
aatgatacggcgaccaccga

SEQ ID NO: 35 - DNA, 18 bp, Artificial Sequence
  HindIII target site
tactcaagcttaccccta

SEQ ID NO: 36 - DNA, 22 bp, Artificial Sequence
  Adaptor Sequence - optionally may be absent
ggaaagcggaggcgtagtggtt

SEQ ID NO: 37 - DNA, 32 bp, Artificial Sequence
  Adaptor Sequence
gatcggaagagcgtcgtgtagggaaagagtgt

SEQ ID NO: 38 - DNA, 21 bp, Artificial Sequence
  Adaptor Sequence
tcggtggtcgccgtatcattc

SEQ ID NO: 39 - DNA, 33 bp, Artificial Sequence
  Adaptor Sequence
acactctttccctacacgacgctcttccgatct

SEQ ID NO: 40 - DNA, 23 bp, Artificial Sequence
  Adaptor Sequence
aacccactacgcctccgctttcc

SEQ ID NO: 41 - DNA, 29 bp, Artificial Sequence
  Adaptor Sequence
aatgatacggcgaccaccgagatctacac

SEQ ID NO: 42 - DNA, 29 bp, Artificial Sequence
  Adaptor Sequence
gtgtagatctcggtggtcgccgtatcatt

SEQ ID NO: 43 - DNA, 18 bp, Artificial Sequence
  HindIII target site
ggggggtaagcttgagta

SEQ ID NO: 44 - DNA, 23 bp, Artificial Sequence
  EMX1 sgRNA target site
  misc_feature (21)..(21): n is a, c, g, or t
gagtccgagcagaagaagaangg

SEQ ID NO: 45 - DNA, 40 bp, Artificial Sequence
  EMX1 ON read
cctgagtccgagcagaagaagaagggctcccatcacatca

SEQ ID NO: 46 - DNA, 40 bp, Artificial Sequence
  EMX1 ON read
cctgagtccgagcagaagaaagaagggctcccatcacatc

SEQ ID NO: 47 - DNA, 40 bp, Artificial Sequence; identical to SEQ ID NO: 45
  EMX1 ON read

SEQ ID NO: 48 - DNA, 34 bp, Artificial Sequence
  EMX1 ON read
cctgagtccgagcagaagggctcccatcacatca

SEQ ID NO: 49 - DNA, 37 bp, Artificial Sequence
  EMX1 ON read
cctgagtccgagcagaagaagggctcccatcacatca

SEQ ID NO: 50 - DNA, 39 bp, Artificial Sequence
  EMX1 ON read
cctgagtccgagcagaagagaagggctcccatcacatca

SEQ ID NO: 51 - DNA, 38 bp, Artificial Sequence
  EMX1 ON read
cctgagtccgagcagaagaaagggctcccatcacatca

SEQ ID NO: 52 - DNA, 40 bp, Artificial Sequence
  EMX1 ON read
cctgagtccgagcagaagaagcagaagggctcccatcaca

SEQ ID NO: 53 - DNA, 29 bp, Artificial Sequence
  EMX1 ON read
cctgagtccgagcagaagggctcccatca

SEQ ID NO: 54 - DNA, 37 bp, Artificial Sequence
  EMX1 ON read
cctgagtccgagcacaggaagggctcccatcacatca

SEQ ID NO: 55 - DNA, 18 bp, Artificial Sequence
  EMX1 ON read
cctgagtccatcacatca

SEQ ID NO: 56 - DNA, 20 bp, Artificial Sequence
  EMX1 ON read
cctgagctcccatcacatca

SEQ ID NO: 57 - DNA, 27 bp, Artificial Sequence
  EMX1 ON read
cctgaaagaagggctcccatcacatca

SEQ ID NO: 58 - DNA, 40 bp, Artificial Sequence
  EMX1 ON read
cctgagtccgagcagaagaagagaagggctcccattacat

SEQ ID NO: 59 - DNA, 36 bp, Artificial Sequence
  EMX1 ON read
cctgagtccgagcagagaagggctcccatcacatca

SEQ ID NO: 60 - DNA, 40 bp, Artificial Sequence
  EMX1 ON read
cctgagtccgagcagaagaaaagaagggctcccatcacat

SEQ ID NO: 61 - DNA, 29 bp, Artificial Sequence
  EMX1 ON read
cctgagtcagaagggctcccatcacatca

SEQ ID NO: 62 - DNA, 40 bp, Artificial Sequence
  EMX1 ON read
cctgagtccgagcagaagaagagaagggctcccatcacat

SEQ ID NO: 63 - DNA, 40 bp, Artificial Sequence
  EMX1 ON read
cctgagtccgagcagaagaagaagaagaagaagaagaaga

SEQ ID NO: 64 - DNA, 40 bp, Artificial Sequence
  EMX1 ON read
cctgagtccgagcggaagaaagaagggctcccatcacatc

SEQ ID NO: 65 - DNA, 18 bp, Artificial Sequence
  EMX1 ON read
cctgctcccatcacatca

SEQ ID NO: 66 - DNA, 40 bp, Artificial Sequence
  EMX1 OT-1 read
tcagagttagagcagaagaagaaaggcatggagtaaaggc

SEQ ID NO: 67 - DNA, 40 bp, Artificial Sequence
  EMX1 OT-1 read
tcagagttagagcagaagaaagaaaggcatggagtaaagg

SEQ ID NO: 68 - DNA, 37 bp, Artificial Sequence
  EMX1 OT-1 read
tcagagttagagcagaagaaaggcatggagtaaaggc

SEQ ID NO: 69 - DNA, 26 bp, Artificial Sequence
  EMX1 OT-1 read
tcagagttagagcatggagtaaaggc

SEQ ID NO: 70 - DNA, 34 bp, Artificial Sequence
  EMX1 OT-1 read
tcagagttagagcagaaaggcatggagtaaaggc

SEQ ID NO: 71 - DNA, 27 bp, Artificial Sequence
  EMX1 OT-1 read
tcagagttagagcagaagagtaaaggc

SEQ ID NO: 72 - DNA, 33 bp, Artificial Sequence
  EMX1 OT-1 read
tcagagttagagcagaaggcatggagtaaaggc

SEQ ID NO: 73 - DNA, 31 bp, Artificial Sequence
  EMX1 OT-1 read
tcagagttagagaaaggcatggagtaaaggc

SEQ ID NO: 74 - DNA, 26 bp, Artificial Sequence
  EMX1 OT-1 read
tcagaagaaaggcatggagtaaaggc

SEQ ID NO: 75 - DNA, 35 bp, Artificial Sequence
  EMX1 OT-1 read
tcagagttagagcagaagaagcatggagtaaaggc

SEQ ID NO: 76 - DNA, 33 bp, Artificial Sequence
  EMX1 OT-1 read
tcagagttagagagaaaggcatggagtaaaggc

SEQ ID NO: 77 - DNA, 36 bp, Artificial Sequence
  EMX1 OT-1 read
tcagagttagagcagagaaaggcatggagtaaaggc

SEQ ID NO: 78 - DNA, 29 bp, Artificial Sequence
  EMX1 OT-1 read
tcagagttagaaaggcatggagtaaaggc

SEQ ID NO: 79 - DNA, 29 bp, Artificial Sequence
  EMX1 OT-1 read
tcagagttagagcagaagaaagtaaaggc

SEQ ID NO: 80 - DNA, 40 bp, Artificial Sequence
  EMX1 OT-1 read
tcagagttagagcagaagaagaaaggtatggagtaaaggc

SEQ ID NO: 81 - DNA, 37 bp, Artificial Sequence
  EMX1 OT-1 read
tcagagttagagcatgagaaaggcatggagtaaaggc

SEQ ID NO: 82 - DNA, 40 bp, Artificial Sequence
  EMX1 OT-1 read
tcagagttagagcagaagaaaagaaaggcatggagtaaag

SEQ ID NO: 83 - DNA, 40 bp, Artificial Sequence
  EMX1 OT-1 read
tcagagttagagcagaagaagaaaggcatggggtaaaggc

SEQ ID NO: 84 - DNA, 40 bp, Artificial Sequence
  EMX1 OT-1 read
tcagagttagagcagaagaaaaccactacctgagcaccca

SEQ ID NO: 85 - DNA, 40 bp, Artificial Sequence
  EMX1 OT-1 read
tcagagttagagcagaagaagaagaaaggcatggagtaaa

SEQ ID NO: 86 - DNA, 40 bp, Artificial Sequence
  EMX1 OT-1 read
tcagagttagagcagaagaactgagcacccagtccgccct

SEQ ID NO: 87 - DNA, 33 bp, Artificial Sequence
  EMX1 OT-1 read
tcagagttagagcagaagaaatggagtaaaggc

SEQ ID NO: 88 - DNA, 40 bp, Artificial Sequence
  EMX1 OT-2 read
caagagtctaagcagaagaagaagagagccactacccaac

SEQ ID NO: 89 - DNA, 40 bp, Artificial Sequence
  EMX1 OT-2 read
caagagtctaagcagaagaaagaagagagccactacccaa

SEQ ID NO: 90 - DNA, 37 bp, Artificial Sequence
  EMX1 OT-2 read
caagagtctaagcagaagaagagagccactacccaac

SEQ ID NO: 91 - DNA, 39 bp, Artificial Sequence
  EMX1 OT-2 read
caagagtctaagcagaagagaagagagccactacccaac

SEQ ID NO: 92 - DNA, 40 bp, Artificial Sequence
  EMX1 OT-2 read
caagagcctaagcagaagaagaagagagccactacccaac

SEQ ID NO: 93 - DNA, 40 bp, Artificial Sequence
  EMX1 OT-2 read
caagagtctaagcagaagaagaggagagccactacccaac

SEQ ID NO: 94 - DNA, 40 bp, Artificial Sequence
  EMX1 OT-2 read
cgagagtctaagcagaagaagaagagagccactacccaac

SEQ ID NO: 95 - DNA, 40 bp, Artificial Sequence
  EMX1 OT-2 read
caagggtctaagcagaagaagaagagagccactacccaac

SEQ ID NO: 96 - DNA, 40 bp, Artificial Sequence
  EMX1 OT-2 read
caagagtctaagcagaagaaggagagagccactacccaac

SEQ ID NO: 97 - DNA, 40 bp, Artificial Sequence
  EMX1 OT-2 read
caagagtctaagcagaggaagaagagagccactacccaac

SEQ ID NO: 98 - DNA, 40 bp, Artificial Sequence
  EMX1 OT-2 read
caagagtctaagcaggagaagaagagagccactacccaac

SEQ ID NO: 99 - DNA, 40 bp, Artificial Sequence
  EMX1 OT-2 read
caagagtctaagcagaagaagaagagggccactacccaac

SEQ ID NO: 100 - DNA, 40 bp, Artificial Sequence
  EMX1 OT-2 read
caagagtctaagcagaagaggaagagagccactacccaac

SEQ ID NO: 101 - DNA, 40 bp, Artificial Sequence
  EMX1 OT-2 read
caagagtctaagcagaaggagaagagagccactacccaac

SEQ ID NO: 102 - DNA, 40 bp, Artificial Sequence
  EMX1 OT-2 read
caggagtctaagcagaagaagaagagagccactacccaac

SEQ ID NO: 103 - DNA, 40 bp, Artificial Sequence
  EMX1 OT-2 read
caagagtctaagcagaagaagaagggagccactacccaac

SEQ ID NO: 104 - DNA, 40 bp, Artificial Sequence
  EMX1 OT-2 read
caagagtctaggcagaagaagaagagagccactacccaac

SEQ ID NO: 105 - DNA, 40 bp, Artificial Sequence
  EMX1 OT-2 read
caagagtctaagcggaagaagaagagagccactacccaac

SEQ ID NO: 106 - DNA, 23 bp, Artificial Sequence
  Primer
ccatctcatccctgcgtgtctcc

SEQ ID NO: 107 - DNA, 44 bp, Artificial Sequence
  Adaptor Sequence
ccatctcatccctgcgtgtctccgactcagctaaggtaacgatt

SEQ ID NO: 108 - DNA, 43 bp, Artificial Sequence
  Adaptor Sequence
atcgttaccttagctgagtcggagacacgcagggatgagatgg

SEQ ID NO: 109 - DNA, 21 bp, Artificial Sequence
  Adaptor Sequence
atcaccgactgcccatagaga

SEQ ID NO: 110 - DNA, 45 bp, Artificial Sequence
  Adaptor Sequence
aacccactacgcctccgctttcctctctatgggcagtcggtgatt

SEQ ID NO: 111 - DNA, 23 bp, Artificial Sequence
  Adaptor Sequence
aacccactacgcctccgctttcc